European Patent Application EP 4 549 572 A1, published May 7, 2025. Title: Fusion proteins. Applicant: 株式会社カイオム・バイオサイエンス. Application JP. The sequence listing filed with the application follows.

SEQUENCE LISTING (109 sequences)

SEQ ID NO: 1 - protein, 482 aa, synthetic construct
  REGION 1..482: note = Recombinant peptide
QVQLVQSGAEVKKPGASVKVSCKASGYSFTSYYMHWVKQSPGQGLEWIGRINPNNGVTLYNQKFKDRVTMTRDTSISTAYMELSRLRSDDTAVYYCARSTMITNYVMDYWGQGTLVTVSSASTKGPSVFPLAPSSKSTSGGTAALGCLVKDYFPEPVTVSWNSGALTSGVHTFPAVLQSSGLYSLSSVVTVPSSSLGTQTYICNVNHKPSNTKVDKKVEPKSCDKTHTGPGGGSPGQVQLVQSGAELKKPGASVKVSCKASGYTFTRYTMHWVRQAPGQCLEWMGYINPSRGYTNYNQKFKDKATLTADKSTSTAYMELRSLRSDDTAVYYCARYYDDHYSLDYWGQGTLVTVSSASGGGGSGGGGSGGGGSAGDIQLTQSPSILSASVGDRVTITCRASSSVSYMNWYQQKPGKAPKRWIYDTSKVASGVPYRFSGSGSGTEYTLTISSMQPEDFATYYCQQWSSNPLTFGCGTKVEIKSG

SEQ ID NO: 2 - protein, 228 aa, synthetic construct
  REGION 1..228: note = Recombinant peptide
QVQLVQSGAEVKKPGASVKVSCKASGYSFTSYYMHWVKQSPGQGLEWIGRINPNNGVTLYNQKFKDRVTMTRDTSISTAYMELSRLRSDDTAVYYCARSTMITNYVMDYWGQGTLVTVSSASTKGPSVFPLAPSSKSTSGGTAALGCLVKDYFPEPVTVSWNSGALTSGVHTFPAVLQSSGLYSLSSVVTVPSSSLGTQTYICNVNHKPSNTKVDKKVEPKSCDKTHT

SEQ ID NO: 3 - protein, 5 aa, synthetic construct
  REGION 1..5: note = Recombinant peptide
SYYMH

SEQ ID NO: 4 - protein, 17 aa, synthetic construct
  REGION 1..17: note = Recombinant peptide
RINPNNGVTLYNQKFKD

SEQ ID NO: 5 - protein, 11 aa, synthetic construct
  REGION 1..11: note = Recombinant peptide
STMITNYVMDY

SEQ ID NO: 6 - protein, 8 aa, synthetic construct
  REGION 1..8: note = Recombinant peptide
GPGGGSPG

SEQ ID NO: 7 - protein, 246 aa, synthetic construct
  REGION 1..246: note = Recombinant peptide
QVQLVQSGAELKKPGASVKVSCKASGYTFTRYTMHWVRQAPGQCLEWMGYINPSRGYTNYNQKFKDKATLTADKSTSTAYMELRSLRSDDTAVYYCARYYDDHYSLDYWGQGTLVTVSSASGGGGSGGGGSGGGGSAGDIQLTQSPSILSASVGDRVTITCRASSSVSYMNWYQQKPGKAPKRWIYDTSKVASGVPYRFSGSGSGTEYTLTISSMQPEDFATYYCQQWSSNPLTFGCGTKVEIKSG

SEQ ID NO: 8 - protein, 121 aa, synthetic construct
  REGION 1..121: note = Recombinant peptide
QVQLVQSGAELKKPGASVKVSCKASGYTFTRYTMHWVRQAPGQCLEWMGYINPSRGYTNYNQKFKDKATLTADKSTSTAYMELRSLRSDDTAVYYCARYYDDHYSLDYWGQGTLVTVSSAS

SEQ ID NO: 9 - protein, 5 aa, synthetic construct
  REGION 1..5: note = Recombinant peptide
RYTMH

SEQ ID NO: 10 - protein, 17 aa, synthetic construct
  REGION 1..17: note = Recombinant peptide
YINPSRGYTNYNQKFKD

SEQ ID NO: 11 - protein, 10 aa, synthetic construct
  REGION 1..10: note = Recombinant peptide
YYDDHYSLDY

SEQ ID NO: 12 - protein, 19 aa, synthetic construct
  REGION 1..19: note = Recombinant peptide
ASGGGGSGGGGSGGGGSAG

SEQ ID NO: 13 - protein, 106 aa, synthetic construct
  REGION 1..106: note = Recombinant peptide
DIQLTQSPSILSASVGDRVTITCRASSSVSYMNWYQQKPGKAPKRWIYDTSKVASGVPYRFSGSGSGTEYTLTISSMQPEDFATYYCQQWSSNPLTFGCGTKVEIK

SEQ ID NO: 14 - protein, 10 aa, synthetic construct
  REGION 1..10: note = Recombinant peptide
RASSSVSYMN

SEQ ID NO: 15 - protein, 7 aa, synthetic construct
  REGION 1..7: note = Recombinant peptide
DTSKVAS

SEQ ID NO: 16 - protein, 9 aa, synthetic construct
  REGION 1..9: note = Recombinant peptide
QQWSSNPLT

SEQ ID NO: 17 - protein, 478 aa, synthetic construct
  REGION 1..478: note = Recombinant peptide
DIVMTQSPDSLAVSLGERATINCKASQSVSNDVAWYQQKPGQPPKLLIYYTSSRYAGVPDRFSGSGSGTDFTLTISSLQAEDVAVYYCQQDYNSPPTFGGGTKLEIKRTVAAPSVFIFPPSDEQLKSGTASVVCLLNNFYPREAKVQWKVDNALQSGNSQESVTEQDSKDSTYSLSSTLTLSKADYEKHKVYACEVTHQGLSSPVTKSFNRGECGPGGGSPGQVQLQESGPGVVKPSGTLSLTCAISGGSIGSGGSIRSTRWWSWVRQSPGKGLEWIGEIYHSGSTNYNPSLKSRVTISLDKSRNHFSLRLNSVTAADTAVYYCARQDYGDSGDWYFDLWGKGTLVTVSSGGGGSGGGGSGGGGSQAVLTQPSSVSGAPGQRVTISCTGSSSNIGAGYDVHWYQQLPGTAPKLLIYGNNNRPSGVPDRFSGSKSGTSASLAITGLQTEDEADYYCQSYDNSLSGEVFGGGTKVTVLSG

SEQ ID NO: 18 - protein, 214 aa, synthetic construct
  REGION 1..214: note = Recombinant peptide
DIVMTQSPDSLAVSLGERATINCKASQSVSNDVAWYQQKPGQPPKLLIYYTSSRYAGVPDRFSGSGSGTDFTLTISSLQAEDVAVYYCQQDYNSPPTFGGGTKLEIKRTVAAPSVFIFPPSDEQLKSGTASVVCLLNNFYPREAKVQWKVDNALQSGNSQESVTEQDSKDSTYSLSSTLTLSKADYEKHKVYACEVTHQGLSSPVTKSFNRGEC

SEQ ID NO: 19 - protein, 11 aa, synthetic construct
  REGION 1..11: note = Recombinant peptide
KASQSVSNDVA

SEQ ID NO: 20 - protein, 7 aa, synthetic construct
  REGION 1..7: note = Recombinant peptide
YTSSRYA

SEQ ID NO: 21 - protein, 9 aa, synthetic construct
  REGION 1..9: note = Recombinant peptide
QQDYNSPPT

SEQ ID NO: 22 - protein, 256 aa, synthetic construct
  REGION 1..256: note = Recombinant peptide
QVQLQESGPGVVKPSGTLSLTCAISGGSIGSGGSIRSTRWWSWVRQSPGKGLEWIGEIYHSGSTNYNPSLKSRVTISLDKSRNHFSLRLNSVTAADTAVYYCARQDYGDSGDWYFDLWGKGTLVTVSSGGGGSGGGGSGGGGSQAVLTQPSSVSGAPGQRVTISCTGSSSNIGAGYDVHWYQQLPGTAPKLLIYGNNNRPSGVPDRFSGSKSGTSASLAITGLQTEDEADYYCQSYDNSLSGEVFGGGTKVTVLSG

SEQ ID NO: 23 - protein, 128 aa, synthetic construct
  REGION 1..128: note = Recombinant peptide
QVQLQESGPGVVKPSGTLSLTCAISGGSIGSGGSIRSTRWWSWVRQSPGKGLEWIGEIYHSGSTNYNPSLKSRVTISLDKSRNHFSLRLNSVTAADTAVYYCARQDYGDSGDWYFDLWGKGTLVTVSS

SEQ ID NO: 24 - protein, 12 aa, synthetic construct
  REGION 1..12: note = Recombinant peptide
SGGSIRSTRWWS

SEQ ID NO: 25 - protein, 16 aa, synthetic construct
  REGION 1..16: note = Recombinant peptide
EIYHSGSTNYNPSLKS

SEQ ID NO: 26 - protein, 13 aa, synthetic construct
  REGION 1..13: note = Recombinant peptide
QDYGDSGDWYFDL

SEQ ID NO: 27 - protein, 13 aa, synthetic construct
  REGION 1..13: note = Recombinant peptide
QDYGSSGDWYFDL

SEQ ID NO: 28 - protein, 111 aa, synthetic construct
  REGION 1..111: note = Recombinant peptide
QAVLTQPSSVSGAPGQRVTISCTGSSSNIGAGYDVHWYQQLPGTAPKLLIYGNNNRPSGVPDRFSGSKSGTSASLAITGLQTEDEADYYCQSYDNSLSGEVFGGGTKVTVL

SEQ ID NO: 29 - protein, 14 aa, synthetic construct
  REGION 1..14: note = Recombinant peptide
TGSSSNIGAGYDVH

SEQ ID NO: 30 - protein, 7 aa, synthetic construct
  REGION 1..7: note = Recombinant peptide
GNNNRPS

SEQ ID NO: 31 - protein, 11 aa, synthetic construct
  REGION 1..11: note = Recombinant peptide
QSYDNSLSGEV

SEQ ID NO: 32 - protein, 11 aa, synthetic construct
  REGION 1..11: note = Recombinant peptide
QSYDASLSGEV

SEQ ID NO: 33 - protein, 11 aa, synthetic construct
  REGION 1..11: note = Recombinant peptide
QSYDNALSGEV

SEQ ID NO: 34 - protein, 478 aa, synthetic construct
  REGION 1..478: note = Recombinant peptide
DIVMTQSPDSLAVSLGERATINCKASQSVSNDVAWYQQKPGQPPKLLIYYTSSRYAGVPDRFSGSGSGTDFTLTISSLQAEDVAVYYCQQDYNSPPTFGGGTKLEIKRTVAAPSVFIFPPSDEQLKSGTASVVCLLNNFYPREAKVQWKVDNALQSGNSQESVTEQDSKDSTYSLSSTLTLSKADYEKHKVYACEVTHQGLSSPVTKSFNRGECGPGGGSPGEVQLLESGGGLVQPGGSLRLSCAASGFTFSSYAMSWVRQAPGKGLEWVSAISGSGGSTYYADSVKGRFTISRDNSKDTLYLQMNSLRAEDTAVYYCARDGPLYDISAGFVPISYYLDYWGQGTTVTVSSGGGGSGGGGSGGGGSQPVLTQPPSASGTPGQRVTISCSGSFSNIGSNYVFWYQQLPGTAPKLLISGNNQRPSGVPDRFSGSKSGTSASLAISGLRSQDEADYYCATWDDSLRGWVFGGGTKLTVLSG

SEQ ID NO: 35 - protein, 256 aa, synthetic construct
  REGION 1..256: note = Recombinant peptide
EVQLLESGGGLVQPGGSLRLSCAASGFTFSSYAMSWVRQAPGKGLEWVSAISGSGGSTYYADSVKGRFTISRDNSKDTLYLQMNSLRAEDTAVYYCARDGPLYDISAGFVPISYYLDYWGQGTTVTVSSGGGGSGGGGSGGGGSQPVLTQPPSASGTPGQRVTISCSGSFSNIGSNYVFWYQQLPGTAPKLLISGNNQRPSGVPDRFSGSKSGTSASLAISGLRSQDEADYYCATWDDSLRGWVFGGGTKLTVLSG

SEQ ID NO: 36 - protein, 129 aa, synthetic construct
  REGION 1..129: note = Recombinant peptide
EVQLLESGGGLVQPGGSLRLSCAASGFTFSSYAMSWVRQAPGKGLEWVSAISGSGGSTYYADSVKGRFTISRDNSKDTLYLQMNSLRAEDTAVYYCARDGPLYDISAGFVPISYYLDYWGQGTTVTVSS

SEQ ID NO: 37 - protein, 5 aa, synthetic construct
  REGION 1..5: note = Recombinant peptide
SYAMS

SEQ ID NO: 38 - protein, 17 aa, synthetic construct
  REGION 1..17: note = Recombinant peptide
AISGSGGSTYYADSVKG

SEQ ID NO: 39 - protein, 20 aa, synthetic construct
  REGION 1..20: note = Recombinant peptide
DGPLYDISAGFVPISYYLDY

SEQ ID NO: 40 - protein, 110 aa, synthetic construct
  REGION 1..110: note = Recombinant peptide
QPVLTQPPSASGTPGQRVTISCSGSFSNIGSNYVFWYQQLPGTAPKLLISGNNQRPSGVPDRFSGSKSGTSASLAISGLRSQDEADYYCATWDDSLRGWVFGGGTKLTVL

SEQ ID NO: 41 - protein, 13 aa, synthetic construct
  REGION 1..13: note = Recombinant peptide
SGSFSNIGSNYVF

SEQ ID NO: 42 - protein, 6 aa, synthetic construct
  REGION 1..6: note = Recombinant peptide
GNNQRP

SEQ ID NO: 43 - protein, 11 aa, synthetic construct
  REGION 1..11: note = Recombinant peptide
ATWDDSLRGWV

SEQ ID NO: 44 - protein, 469 aa, synthetic construct
  REGION 1..469: note = Recombinant peptide
DIVMTQSPDSLAVSLGERATINCKASQSVSNDVAWYQQKPGQPPKLLIYYTSSRYAGVPDRFSGSGSGTDFTLTISSLQAEDVAVYYCQQDYNSPPTFGGGTKLEIKRTVAAPSVFIFPPSDEQLKSGTASVVCLLNNFYPREAKVQWKVDNALQSGNSQESVTEQDSKDSTYSLSSTLTLSKADYEKHKVYACEVTHQGLSSPVTKSFNRGECGPGGGSPGEVQLLESGGGLVQPGGSLRLSCAASGFTFSSYAMSWVRQAPGKGLEWVSAISGSGGSTYYADSVKGRFTISRDNSKNTLYLQMNSLRAEDTAVYYCARTKWELVDPYDYWGQGTMVTVSSGGGGSGGGGSGGGGSNFMLTQPHSVSESPGKTITISCTRSSGSIAGNYVQWYQQRPGSAPIIVIYEDNQRPSGVPDRFSGSIDSSSNSASLTISRLKTEDEADYYCQSYEASNVVFGGGTKLTVLSG

SEQ ID NO: 45 - protein, 247 aa, synthetic construct
  REGION 1..247: note = Recombinant peptide
EVQLLESGGGLVQPGGSLRLSCAASGFTFSSYAMSWVRQAPGKGLEWVSAISGSGGSTYYADSVKGRFTISRDNSKNTLYLQMNSLRAEDTAVYYCARTKWELVDPYDYWGQGTMVTVSSGGGGSGGGGSGGGGSNFMLTQPHSVSESPGKTITISCTRSSGSIAGNYVQWYQQRPGSAPIIVIYEDNQRPSGVPDRFSGSIDSSSNSASLTISRLKTEDEADYYCQSYEASNVVFGGGTKLTVLSG

SEQ ID NO: 46 - protein, 120 aa, synthetic construct
  REGION 1..120: note = Recombinant peptide
EVQLLESGGGLVQPGGSLRLSCAASGFTFSSYAMSWVRQAPGKGLEWVSAISGSGGSTYYADSVKGRFTISRDNSKNTLYLQMNSLRAEDTAVYYCARTKWELVDPYDYWGQGTMVTVSS

SEQ ID NO: 47 - protein, 5 aa, synthetic construct
  REGION 1..5: note = Recombinant peptide
SYAMS

SEQ ID NO: 48 - protein, 17 aa, synthetic construct
  REGION 1..17: note = Recombinant peptide
AISGSGGSTYYADSVKG

SEQ ID NO: 49 - protein, 17 aa, synthetic construct
  REGION 1..17: note = Recombinant peptide
AISGSGGSTYYASSVKG

SEQ ID NO: 50 - protein, 11 aa, synthetic construct
  REGION 1..11: note = Recombinant peptide
TKWELVDPYDY

SEQ ID NO: 51 - protein, 110 aa, synthetic construct
  REGION 1..110: note = Recombinant peptide
NFMLTQPHSVSESPGKTITISCTRSSGSIAGNYVQWYQQRPGSAPIIVIYEDNQRPSGVPDRFSGSIDSSSNSASLTISRLKTEDEADYYCQSYEASNVVFGGGTKLTVL

SEQ ID NO: 52 - protein, 13 aa, synthetic construct
  REGION 1..13: note = Recombinant peptide
TRSSGSIAGNYVQ

SEQ ID NO: 53 - protein, 7 aa, synthetic construct
  REGION 1..7: note = Recombinant peptide
EDNQRPS

SEQ ID NO: 54 - protein, 9 aa, synthetic construct
  REGION 1..9: note = Recombinant peptide
QSYEASNVV

SEQ ID NO: 55 - protein, 469 aa, synthetic construct
  REGION 1..469: note = Recombinant peptide
DIVMTQSPDSLAVSLGERATINCKASQSVSNDVAWYQQKPGQPPKLLIYYTSSRYAGVPDRFSGSGSGTDFTLTISSLQAEDVAVYYCQQDYNSPPTFGGGTKLEIKRTVAAPSVFIFPPSDEQLKSGTASVVCLLNNFYPREAKVQWKVDNALQSGNSQESVTEQDSKDSTYSLSSTLTLSKADYEKHKVYACEVTHQGLSSPVTKSFNRGECGPGGGSPGEVQLLESGGGLVQPGGSLRLSCAASGFTFSSYAMSWVRQAPGKGLEWVSAISGSGGSTYYADSVKGRFTISRDNSKNTLYLQMNSLRAEDTAVYYCARSKWELVDPYGNWGQGTMVTVSSGGGGSGGGGSGGGGSNFMLTQPHSVSESPGKTITISCTRSSGSIAGNYVQWYQQRPGSAPIIVIYEDNQRPSGVPDRFSGSIDSSSNSASLTISRLKTEDEADYYCQSYEASNVVFGGGTKLTVLSG

SEQ ID NO: 56 - protein, 247 aa, synthetic construct
  REGION 1..247: note = Recombinant peptide
EVQLLESGGGLVQPGGSLRLSCAASGFTFSSYAMSWVRQAPGKGLEWVSAISGSGGSTYYADSVKGRFTISRDNSKNTLYLQMNSLRAEDTAVYYCARSKWELVDPYGNWGQGTMVTVSSGGGGSGGGGSGGGGSNFMLTQPHSVSESPGKTITISCTRSSGSIAGNYVQWYQQRPGSAPIIVIYEDNQRPSGVPDRFSGSIDSSSNSASLTISRLKTEDEADYYCQSYEASNVVFGGGTKLTVLSG

SEQ ID NO: 57 - protein, 120 aa, synthetic construct
  REGION 1..120: note = Recombinant peptide
EVQLLESGGGLVQPGGSLRLSCAASGFTFSSYAMSWVRQAPGKGLEWVSAISGSGGSTYYADSVKGRFTISRDNSKNTLYLQMNSLRAEDTAVYYCARSKWELVDPYGNWGQGTMVTVSS

SEQ ID NO: 58 - protein, 5 aa, synthetic construct
  REGION 1..5: note = Recombinant peptide
SYAMS

SEQ ID NO: 59 - protein, 17 aa, synthetic construct
  REGION 1..17: note = Recombinant peptide
AISGSGGSTYYADSVKG

SEQ ID NO: 60 - protein, 11 aa, synthetic construct
  REGION 1..11: note = Recombinant peptide
SKWELVDPYGN

SEQ ID NO: 61 - protein, 110 aa, synthetic construct; identical to SEQ ID NO: 51
  REGION 1..110: note = Recombinant peptide

SEQ ID NO: 62 - protein, 13 aa, synthetic construct
  REGION 1..13: note = Recombinant peptide
TRSSGSIAGNYVQ

SEQ ID NO: 63 - protein, 7 aa, synthetic construct
  REGION 1..7: note = Recombinant peptide
EDNQRPS

SEQ ID NO: 64 - protein, 9 aa, synthetic construct
  REGION 1..9: note = Recombinant peptide
QSYEASNVV

SEQ ID NO: 65 - protein, 469 aa, synthetic construct
  REGION 1..469: note = Recombinant peptide
DIVMTQSPDSLAVSLGERATINCKASQSVSNDVAWYQQKPGQPPKLLIYYTSSRYAGVPDRFSGSGSGTDFTLTISSLQAEDVAVYYCQQDYNSPPTFGGGTKLEIKRTVAAPSVFIFPPSDEQLKSGTASVVCLLNNFYPREAKVQWKVDNALQSGNSQESVTEQDSKDSTYSLSSTLTLSKADYEKHKVYACEVTHQGLSSPVTKSFNRGECGPGGGSPGQVTLRESGPALVKPTQTLTLTCTFSGFSLSTSGMSVGWIRQPPGKALEWLADIWWDDKKDYNPSLKSRLTISKDTSKNQVVLKVTNMDPADTATYYCARSMITNWYFDVWGAGTTVTVSSASGGGGSGGGGSGGGGSAGDIQMTQSPSTLSASVGDRVTITCKCQLSVGYMHWYQQKPGKAPKLLIYDTSKLASGVPSRFSGSGSGTEFTLTISSLQPDDFATYYCFQGSGYPFTFGGGTKLEIKSG

SEQ ID NO: 66 - protein, 247 aa, synthetic construct
  REGION 1..247: note = Recombinant peptide
QVTLRESGPALVKPTQTLTLTCTFSGFSLSTSGMSVGWIRQPPGKALEWLADIWWDDKKDYNPSLKSRLTISKDTSKNQVVLKVTNMDPADTATYYCARSMITNWYFDVWGAGTTVTVSSASGGGGSGGGGSGGGGSAGDIQMTQSPSTLSASVGDRVTITCKCQLSVGYMHWYQQKPGKAPKLLIYDTSKLASGVPSRFSGSGSGTEFTLTISSLQPDDFATYYCFQGSGYPFTFGGGTKLEIKSG

SEQ ID NO: 67 - protein, 120 aa, synthetic construct
  REGION 1..120: note = Recombinant peptide
QVTLRESGPALVKPTQTLTLTCTFSGFSLSTSGMSVGWIRQPPGKALEWLADIWWDDKKDYNPSLKSRLTISKDTSKNQVVLKVTNMDPADTATYYCARSMITNWYFDVWGAGTTVTVSS

SEQ ID NO: 68 - protein, 7 aa, synthetic construct
  REGION 1..7: note = Recombinant peptide
TSGMSVG

SEQ ID NO: 69 - protein, 16 aa, synthetic construct
  REGION 1..16: note = Recombinant peptide
DIWWDDKKDYNPSLKS

SEQ ID NO: 70 - protein, 10 aa, synthetic construct
  REGION 1..10: note = Recombinant peptide
SMITNWYFDV

SEQ ID NO: 71 - protein, 106 aa, synthetic construct
  REGION 1..106: note = Recombinant peptide
DIQMTQSPSTLSASVGDRVTITCKCQLSVGYMHWYQQKPGKAPKLLIYDTSKLASGVPSRFSGSGSGTEFTLTISSLQPDDFATYYCFQGSGYPFTFGGGTKLEIK

SEQ ID NO: 72 - protein, 10 aa, synthetic construct
  REGION 1..10: note = Recombinant peptide
KCQLSVGYMH

SEQ ID NO: 73 - protein, 7 aa, synthetic construct
  REGION 1..7: note = Recombinant peptide
DTSKLAS

SEQ ID NO: 74 - protein, 9 aa, synthetic construct
  REGION 1..9: note = Recombinant peptide
FQGSGYPFT

SEQ ID NO: 75 - protein, 247 aa, synthetic construct
  REGION 1..247: note = Recombinant peptide
EVQLLESGGGLVQPGGSLRLSCAASGFTFSSYAMSWVRQAPGKCLEWVSAISGSGGSTYYADSVKGRFTISRDNSKNTLYLQMNSLRAEDTAVYYCARSKWELVDPYGNWGQGTMVTVSSGGGGSGGGGSGGGGSNFMLTQPHSVSESPGKTITISCTRSSGSIAGNYVQWYQQRPGSAPIIVIYEDNQRPSGVPDRFSGSIDSSSNSASLTISRLKTEDEADYYCQSYEASNVVFGCGTKLTVLSG

SEQ ID NO: 76 - protein, 247 aa, synthetic construct
  REGION 1..247: note = Recombinant peptide
EVQLLESGGGLVQPGGSLRLSCAASGFTFSSYAMSWVRQAPGKCLEWVSAISGSGGSTYYADSVKGRFTISRDNSKNTLYLQMNSLRAEDTAVYYCARSKWELVDPYGNWGQGTMVTVSSGGGGSGGGGSGGGGSNFMLTQPHSVSESPGKTITISCTRSSGSIAGNYVQWYQQRPGSAPIIVIYEDNQRPSGVPDRFSGSIDSSSNSASLTISRLKTEDEADYYCQSYEASNVVFGGCTKLTVLSG

SEQ ID NO: 77 - protein, 247 aa, synthetic construct
  REGION 1..247: note = Recombinant peptide
EVQLLESGGGLVQPGGSLRLSCAASGFTFSSYAMSWVRQAPGKGLEWVSAISGSGGSTYYADSVKGRFTISRDNSKNTLYLQMNSLRAEDTAVYYCARSKWELVDPYGNWGCGTMVTVSSGGGGSGGGGSGGGGSNFMLTQPHSVSESPGKTITISCTRSSGSIAGNYVQWYQQRPGCAPIIVIYEDNQRPSGVPDRFSGSIDSSSNSASLTISRLKTEDEADYYCQSYEASNVVFGGGTKLTVLSG

SEQ ID NO: 78 - protein, 128 aa, synthetic construct
  REGION 1..128: note = Recombinant peptide
QVQLQESGPGVVKPSGTLSLTCAISGGSIGSGGSIRSTRWWSWVRQSPGKGLEWIGEIYHSGSTNYNPSLKSRVTISLDKSRNHFSLRLNSVTAADTAVYYCARQDYGSSGDWYFDLWGKGTLVTVSS

SEQ ID NO: 79 - protein, 111 aa, synthetic construct
  REGION 1..111: note = Recombinant peptide
QAVLTQPSSVSGAPGQRVTISCTGSSSNIGAGYDVHWYQQLPGTAPKLLIYGNNNRPSGVPDRFSGSKSGTSASLAITGLQTEDEADYYCQSYDASLSGEVFGGGTKVTVL

SEQ ID NO: 80 - protein, 111 aa, synthetic construct
  REGION 1..111: note = Recombinant peptide
QAVLTQPSSVSGAPGQRVTISCTGSSSNIGAGYDVHWYQQLPGTAPKLLIYGNNNRPSGVPDRFSGSKSGTSASLAITGLQTEDEADYYCQSYDNALSGEVFGGGTKVTVL

SEQ ID NO: 81 - protein, 120 aa, synthetic construct
  REGION 1..120: note = Recombinant peptide
EVQLLESGGGLVQPGGSLRLSCAASGFTFSSYAMSWVRQAPGKGLEWVSAISGSGGSTYYASSVKGRFTISRDNSKNTLYLQMNSLRAEDTAVYYCARTKWELVDPYDYWGQGTMVTVSS

SEQ ID NO: 82 - protein, 120 aa, synthetic construct
  REGION 1..120: note = Recombinant peptide
EVQLLESGGGLVQPGGSLRLSCAASGFTFSSYAMSWVRQAPGKGLEWVSAISGSGGSTYYASSVKGRFTISRDNSKNTLYLQMNSLRAEDTAVYYCARSKWELVDPYGNWGQGTMVTVSS

SEQ ID NO: 83 - protein, 120 aa, synthetic construct
  REGION 1..120: note = Recombinant peptide
EVQLLESGGGLVQPGGSLRLSCAASGFTFSSYAMSWVRQAPGKCLEWVSAISGSGGSTYYADSVKGRFTISRDNSKNTLYLQMNSLRAEDTAVYYCARSKWELVDPYGNWGQGTMVTVSS

SEQ ID NO: 84 - protein, 120 aa, synthetic construct
  REGION 1..120: note = Recombinant peptide
EVQLLESGGGLVQPGGSLRLSCAASGFTFSSYAMSWVRQAPGKGLEWVSAISGSGGSTYYADSVKGRFTISRDNSKNTLYLQMNSLRAEDTAVYYCARSKWELVDPYGNWGCGTMVTVSS

SEQ ID NO: 85 - protein, 110 aa, synthetic construct
  REGION 1..110: note = Recombinant peptide
NFMLTQPHSVSESPGKTITISCTRSSGSIAGNYVQWYQQRPGSAPIIVIYEDNQRPSGVPDRFSGSIDSSSNSASLTISRLKTEDEADYYCQSYEASNVVFGCGTKLTVL

SEQ ID NO: 86 - protein, 110 aa, synthetic construct
  REGION 1..110: note = Recombinant peptide
NFMLTQPHSVSESPGKTITISCTRSSGSIAGNYVQWYQQRPGSAPIIVIYEDNQRPSGVPDRFSGSIDSSSNSASLTISRLKTEDEADYYCQSYEASNVVFGGCTKLTVL

SEQ ID NO: 87 - protein, 110 aa, synthetic construct
  REGION 1..110: note = Recombinant peptide
NFMLTQPHSVSESPGKTITISCTRSSGSIAGNYVQWYQQRPGCAPIIVIYEDNQRPSGVPDRFSGSIDSSSNSASLTISRLKTEDEADYYCQSYEASNVVFGGGTKLTVL

SEQ ID NO: 88 - protein, 120 aa, synthetic construct
  REGION 1..120: note = Recombinant peptide
QVQLVQSGAEVKKPGASVKVSCKASGYSFTSYYMHWVKQSPGQGLEWIGRINPNNGVTLYNQKFKDRVTMTRDTSISTAYMELSRLRSDDTAVYYCARSTMITNYVMDYWGQGTLVTVSS

SEQ ID NO: 89 - protein, 107 aa, synthetic construct
  REGION 1..107: note = Recombinant peptide
DIVMTQSPDSLAVSLGERATINCKASQSVSNDVAWYQQKPGQPPKLLIYYTSSRYAGVPDRFSGSGSGTDFTLTISSLQAEDVAVYYCQQDYNSPPTFGGGTKLEIK

SEQ ID NO: 90 - protein, 120 aa, synthetic construct
  REGION 1..120: note = Recombinant peptide
QVQLVQSGAEVKKPGASVKVSCKASGYSFTSYYMHWVKQSPGQCLEWIGRINPNNGVTLYNQKFKDRVTMTRDTSISTAYMELSRLRSDDTAVYYCARSTMITNYVMDYWGQGTLVTVSS

SEQ ID NO: 91 - protein, 107 aa, synthetic construct
  REGION 1..107: note = Recombinant peptide
DIVMTQSPDSLAVSLGERATINCKASQSVSNDVAWYQQKPGQPPKLLIYYTSSRYAGVPDRFSGSGSGTDFTLTISSLQAEDVAVYYCQQDYNSPPTFGCGTKLEIK

SEQ ID NO: 92 - protein, 119 aa, synthetic construct
  REGION 1..119: note = Recombinant peptide
QVQLVQSGAELKKPGASVKVSCKASGYTFTRYTMHWVRQAPGQGLEWMGYINPSRGYTNYNQKFKDKATLTADKSTSTAYMELRSLRSDDTAVYYCARYYDDHYSLDYWGQGTLVTVSS

SEQ ID NO: 93 - protein, 106 aa, synthetic construct
  REGION 1..106: note = Recombinant peptide
DIQLTQSPSILSASVGDRVTITCRASSSVSYMNWYQQKPGKAPKRWIYDTSKVASGVPYRFSGSGSGTEYTLTISSMQPEDFATYYCQQWSSNPLTFGGGTKVEIK

SEQ ID NO: 94 - protein, 108 aa, synthetic construct
  REGION 1..108: note = Recombinant peptide
ASTKGPSVFPLAPSSKSTSGGTAALGCLVKDYFPEPVTVSWNSGALTSGVHTFPAVLQSSGLYSLSSVVTVPSSSLGTQTYICNVNHKPSNTKVDKKVEPKSCDKTHT

SEQ ID NO: 95 - protein, 107 aa, synthetic construct [sequence omitted]

SEQ ID NO: 96 - protein, 420 aa, Homo sapiens
MPGGCSRGPAAGDGRLRLARLALVLLGWVSSSSPTSSASSFSSSAPFLASAVSAQPPLPDQCPALCECSEAARTVKCVNRNLTEVPTDLPAYVRNLFLTGNQLAVLPAGAFARRPPLAELAALNLSGSRLDEVRAGAFEHLPSLRQLDLSHNPLADLSPFAFSGSNASVSAPSPLVELILNHIVPPEDERQNRSFEGMVVAALLAGRALQGLRRLELASNHFLYLPRDVLAQLPSLRHLDLSNNSLVSLTYVSFRNLTHLESLHLEDNALKVLHNGTLAELQGLPHIRVFLDNNPWVCDCHMADMVTWLKETEVVQGKDRLTCAYPEKMRNRVLLELNSADLDCDPILPPSLQTSYVFLGIVLALIGAIFLLVLYLNRKGIKKWMHNIRDACRDHMEGYHYRYEINADPRLTNLSSNSDV

SEQ ID NO: 97 - protein, 207 aa, Homo sapiens
MQSGTHWRVLGLCLLSVGVWGQDGNEEMGGITQTPYKVSISGTTVILTCPQYPGSEILWQHNDKNIGGDEDDKNIGSDEDHLSLKEFSELEQSGYYVCYPRGSKPEDANFYLYLRARVCENCMEMDVMSVATIVIVDICITGGLLLLVYYWSKNRKAKAKPVTRGAGAGGRQRGQNKERPPPVPNPDYEPIRKGQRDLYSGLNQRRI

SEQ ID NO: 98 - protein, 171 aa, Homo sapiens
MEHSTFLSGLVLATLLSQVSPFKIPIEELEDRVFVNCNTSITWVEGTVGTLLSDITRLDLGKRILDPRGIYRCNGTDIYKDKESTVQVHYRMCQSCVELDPATVAGIIVTDVIATLLLALGVFCFAGHETGRLSGAADTQALLRNDQVYQPLRDRDDAQYSHLGGNWARNK

SEQ ID NO: 99 - protein, 127 aa, Homo sapiens
MEHSTFLSGLVLATLLSQVSPFKIPIEELEDRVFVNCNTSITWVEGTVGTLLSDITRLDLGKRILDPRGIYRCNGTDIYKDKESTVQVHYRTADTQALLRNDQVYQPLRDRDDAQYSHLGGNWARNK

SEQ ID NO: 100 - protein, 287 aa, Homo sapiens
MQIPQAPWPVVWAVLQLGWRPGWFLDSPDRPWNPPTFSPALLVVTEGDNATFTCSFSNTSESFVLNWYRMSPSNQTDKLAAFPEDRSQPGQDCRFRVTQLPNGRDFHMSVVRARRNDSGTYLCGAISLAPKAQIKESLRAELRVTERRAEVPTAHPSPSPRPAGQFQTLVVGVVGGLLGSLVLLVWVLAVICSRAARGTIGARRTGQPLKEDPSAVPVFSVDYGELDFQWREKTPEPPVPCVPEQTEYATIVFPSGMGTSSPARRGSADGPRSAQPLRPEDGHCSWP

SEQ ID NO: 101 - protein, 290 aa, Homo sapiens
MRIFAVFIFMTYWHLLNAFTVTVPKDLYVVEYGSNMTIECKFPVEKQLDLAALIVYWEMEDKNIIQFVHGEEDLKVQHSSYRQRARLLKDQLSLGNAALQITDVKLQDAGVYRCMISYGGADYKRITVKVNAPYNKINQRILVVDPVTSEHELTCQAEGYPKAEVIWTSSDHQVLSGKTTTTNSKREEKLFNVTSTLRINTTTNEIFYCTFRRLDPEENHTAELVIPELPLAHPPNERTHLVILGAILLCLGVALTFIFRLRKGRMMDVKKCGIQDTNSKKQSDTHLEET

SEQ ID NO: 102 - protein, 176 aa, Homo sapiens
MRIFAVFIFMTYWHLLNAPYNKINQRILVVDPVTSEHELTCQAEGYPKAEVIWTSSDHQVLSGKTTTTNSKREEKLFNVTSTLRINTTTNEIFYCTFRRLDPEENHTAELVIPELPLAHPPNERTHLVILGAILLCLGVALTFIFRLRKGRMMDVKKCGIQDTNSKKQSDTHLEET

SEQ ID NO: 103 - protein, 178 aa, Homo sapiens
MRIFAVFIFMTYWHLLNAFTVTVPKDLYVVEYGSNMTIECKFPVEKQLDLAALIVYWEMEDKNIIQFVHGEEDLKVQHSSYRQRARLLKDQLSLGNAALQITDVKLQDAGVYRCMISYGGADYKRITVKVNAPYNKINQRILVVDPVTSEHELTCQAEGYPKAEVIWTSSDHQVLSGD

SEQ ID NO: 104 - protein, 525 aa, Homo sapiens
MWEAQFLGLLFLQPLWVAPVKPLQPGAEVPVVWAQEGAPAQLPCSPTIPLQDLSLLRRAGVTWQHQPDSGPPAAAPGHPLAPGPHPAAPSSWGPRPRRYTVLSVGPGGLRSGRLPLQPRVQLDERGRQRGDFSLWLRPARRADAGEYRAAVHLRDRALSCRLRLRLGQASMTASPPGSLRASDWVILNCSFSRPDRPASVHWFRNRGQGRVPVRESPHHHLAESFLFLPQVSPMDSGPWGCILTYRDGFNVSIMYNLTVLGLEPPTPLTVYAGAGSRVGLPCRLPAGVGTRSFLTAKWTPPGGGPDLLVTGDNGDFTLRLEDVSQAQAGTYTCHIHLQEQQLNATVTLAIITVTPKSFGSPGSLGKLLCEVTPVSGQERFVWSSLDTPSQRSFSGPWLEAQEAQLLSQPWQCQLYQGERLLGAAVYFTELSSPGAQRSGRAPGALPAGHLLLFLILGVLSLLLLVTGAFGFHLWRRQWRPRRFSALEQGIHPPQAQSKIEELEQEPEPEPEPEPEPEPEPEPEQL

SEQ ID NO: 105 - protein, 360 aa, Homo sapiens
MWEAQFLGLLFLQPLWVAPVKPLQPGAEVPVVWAQEGAPAQLPCSPTIPLQDLSLLRRAGVTWQHQPDSGPPAAAPGHPLAPGPHPAAPSSWGPRPRRYTVLSVGPGGLRSGRLPLQPRVQLDERGRQRGDFSLWLRPARRADAGEYRAAVHLRDRALSCRLRLRLGQASMTASPPGSLRASDWVILNCSFSRPDRPASVHWFRNRGQGRVPVRESPHHHLAESFLFLPQVSPMDSGPWGCILTYRDGFNVSIMYNLTVLGLEPPTPLTVYAGAGSRVGLPCRLPAGVGTRSFLTAKWTPPGGGPDLLVTGDNGDFTLRLEDVSQAQAGTYTCHIHLQEQQLNATVTLAIITGQPQVGKE

SEQ ID NO: 106 - protein, 15 aa, synthetic construct
  REGION 1..15: note = Recombinant peptide
GGGGSGGGGSGGGGS

SEQ ID NO: 107 - protein, 469 aa, synthetic construct
  REGION 1..469: note = Recombinant peptide
DIVMTQSPDSLAVSLGERATINCKASQSVSNDVAWYQQKPGQPPKLLIYYTSSRYAGVPDRFSGSGSGTDFTLTISSLQAEDVAVYYCQQDYNSPPTFGGGTKLEIKRTVAAPSVFIFPPSDEQLKSGTASVVCLLNNFYPREAKVQWKVDNALQSGNSQESVTEQDSKDSTYSLSSTLTLSKADYEKHKVYACEVTHQGLSSPVTKSFNRGECGPGGGSPGEVQLLESGGGLVQPGGSLRLSCAASGFTFSSYAMSWVRQAPGKGLEWVSAISGSGGSTYYASSVKGRFTISRDNSKNTLYLQMNSLRAEDTAVYYCARSKWELVDPYGNWGQGTMVTVSSGGGGSGGGGSGGGGSNFMLTQPHSVSESPGKTITISCTRSSGSIAGNYVQWYQQRPGSAPIIVIYEDNQRPSGVPDRFSGSIDSSSNSASLTISRLKTEDEADYYCQSYEASNVVFGGGTKLTVLSG

SEQ ID NO: 108 - protein, 247 aa, synthetic construct
  REGION 1..247: note = Recombinant peptide
EVQLLESGGGLVQPGGSLRLSCAASGFTFSSYAMSWVRQAPGKGLEWVSAISGSGGSTYYASSVKGRFTISRDNSKNTLYLQMNSLRAEDTAVYYCARSKWELVDPYGNWGQGTMVTVSSGGGGSGGGGSGGGGSNFMLTQPHSVSESPGKTITISCTRSSGSIAGNYVQWYQQRPGSAPIIVIYEDNQRPSGVPDRFSGSIDSSSNSASLTISRLKTEDEADYYCQSYEASNVVFGGGTKLTVLSG

SEQ ID NO: 109 - protein, 120 aa, synthetic construct; identical to SEQ ID NO: 82
  REGION 1..120: note = Recombinant peptide